European Patent Specification EP 4 081 534 B1, published June 28, 2023. Title: PROTECTIVE STAPHYLOCOCCAL EXOTOXIN VACCINE. Applicant: Biomedizinische Forschung & Bio-Produkte AG. The sequence listing filed with the application follows.

SEQUENCE LISTING (38 sequences)

SEQ ID NO: 1 - protein, 239 aa, Staphylococcus aureus
ESQPDPKPDELHKSSKFTGLMENMKVLYDDNHVSAINVKSIDQFLYFDLIYSIKDTKLGNYDNVRVEFKNKDLADKYKDKYVDVFGANYYYQCYFSKKTNDINSHQTDKRKTCMYGGVTEHNGNQLDKYRSITVRVFEDGKNLLSFDVQTNKKKVTAQELDYLTRHYLVKNKKLYEFNNSPYETGYIKFIENENSFWYDMMPAPGDKFDQSKYLMMYNDNKMVDSKDVKIEVYLTTKKK

SEQ ID NO: 2 - DNA, 717 bp, Staphylococcus aureus
gagagtcaaccagatcctaaaccagatgagttgcacaaatcgagtaaattcactggtttgatggaaaatatgaaagttttgtatgatgataatcatgtatcagcaataaacgttaaatctatagatcaatttctatactttgacttaatatattctattaaggacactaagttagggaattatgataatgttcgagtcgaatttaaaaacaaagatttagctgataaatacaaagataaatacgtagatgtgtttggagctaattattattatcaatgttatttttctaaaaaaacgaatgatattaattcgcatcaaactgacaaacgaaaaacttgtatgtatggtggtgtaactgagcataatggaaaccaattagataaatatagaagtattactgttcgggtatttgaagatggtaaaaatttattatcttttgacgtacaaactaataagaaaaaggtgactgctcaagaattagattacctaactcgtcactatttggtgaaaaataaaaaactctatgaatttaacaactcgccttatgaaacgggatatattaaatttatagaaaatgagaatagcttttggtatgacatgatgcctgcaccaggagataaatttgaccaatctaaatatttaatgatgtacaatgacaataaaatggttgattctaaagatgtgaagattgaagtttatcttacgacaaagaaaaag

SEQ ID NO: 3 - protein, 236 aa, Artificial Sequence
  Mutant SEB
ESQPDPKPDELHKSSKFTGLMKVLYDDNHVSAINVKSIDQFLYFDLIYSIKDTKLGNYDNVRVEFKNKDLADKYKDKYVDVFGANYYYQCYFSKKTNDINSHQTDKRKTCMYGGVTEHNGNQLDKYRSITVRVFEDGKNLLSFDVQTNKKKVTAQELDYLTRHYLVKNKKLYEFNNSPYETGYIKFIENENSFWYDMMPAPGDKFDQSKYLMMYNDNKMVDSKDVKIEVYLTTKKK

SEQ ID NO: 4 - DNA, 708 bp, Artificial Sequence
  Mutant SEB
gagagtcaaccagatcctaaaccagatgagttgcacaaatcgagtaaattcactggtttgatgaaagttttgtatgatgataatcatgtatcagcaataaacgttaaatctatagatcaatttctatactttgacttaatatattctattaaggacactaagttagggaattatgataatgttcgagtcgaatttaaaaacaaagatttagctgataaatacaaagataaatacgtagatgtgtttggagctaattattattatcaatgttatttttctaaaaaaacgaatgatattaattcgcatcaaactgacaaacgaaaaacttgtatgtatggtggtgtaactgagcataatggaaaccaattagataaatatagaagtattactgttcgggtatttgaagatggtaaaaatttattatcttttgacgtacaaactaataagaaaaaggtgactgctcaagaattagattacctaactcgtcactatttggtgaaaaataaaaaactctatgaatttaacaactcgccttatgaaacgggatatattaaatttatagaaaatgagaatagcttttggtatgacatgatgcctgcaccaggagataaatttgaccaatctaaatatttaatgatgtacaatgacaataaaatggttgattctaaagatgtgaagattgaagtttatcttacgacaaagaaaaag

SEQ ID NO: 5 - protein, 236 aa, Artificial Sequence
  Mutant SEB
ESQPDPKPDELHKSSKFTGLMKVLYDDNHVSAINVKSIDQFRYFDLIYSIKDTKLGNYDNVRVEFKNKDLADKYKDKYVDVFGANYYYQCYFSKKTNDINSHQTDKRKTCMYGGVTEHNGNQLDKYRSITVRVFEDGKNLLSFDVQTNKKKVTAQELDYLTRHYLVKNKKLYEFNNSPYETGYIKFIENENSFWYDMMPAPGDKFDQSKYLMMYNDNKMVDSKDVKIEVYLTTKKK

SEQ ID NO: 6 - DNA, 708 bp, Artificial Sequence
  Mutant SEB
gagagtcaaccagatcctaaaccagatgagttgcacaaatcgagtaaattcactggtttgatgaaagttttgtatgatgataatcatgtatcagcaataaacgttaaatctatagatcaatttagatactttgacttaatatattctattaaggacactaagttagggaattatgataatgttcgagtcgaatttaaaaacaaagatttagctgataaatacaaagataaatacgtagatgtgtttggagctaattattattatcaatgttatttttctaaaaaaacgaatgatattaattcgcatcaaactgacaaacgaaaaacttgtatgtatggtggtgtaactgagcataatggaaaccaattagataaatatagaagtattactgttcgggtatttgaagatggtaaaaatttattatcttttgacgtacaaactaataagaaaaaggtgactgctcaagaattagattacctaactcgtcactatttggtgaaaaataaaaaactctatgaatttaacaactcgccttatgaaacgggatatattaaatttatagaaaatgagaatagcttttggtatgacatgatgcctgcaccaggagataaatttgaccaatctaaatatttaatgatgtacaatgacaataaaatggttgattctaaagatgtgaagattgaagtttatcttacgacaaagaaaaag

SEQ ID NO: 7 - protein, 236 aa, Artificial Sequence
  Mutant SEB
ESQPDPKPDELHKSSKFTGLMKVLYDDNHVSAINVKSIDPFLYFDLIYSIKDTKLGNYDNVRVEFKNKDLADKYKDKYVDVFGANYYYQCYFSKKTNDINSHQTDKRKTCMYGGVTEHNGNQLDKYRSITVRVFEDGKNLLSFDVQTNKKKVTAQELDYLTRHYLVKNKKLYEFNNSPYETGYIKFIENENSFWYDMMPAPGDKFDQSKYLMMYNDNKMVDSKDVKIEVYLTTKKK

SEQ ID NO: 8 - DNA, 708 bp, Artificial Sequence
  Mutant SEB
gagagtcaaccagatcctaaaccagatgagttgcacaaatcgagtaaattcactggtttgatgaaagttttgtatgatgataatcatgtatcagcaataaacgttaaatctatagatccgtttctatactttgacttaatatattctattaaggacactaagttagggaattatgataatgttcgagtcgaatttaaaaacaaagatttagctgataaatacaaagataaatacgtagatgtgtttggagctaattattattatcaatgttatttttctaaaaaaacgaatgatattaattcgcatcaaactgacaaacgaaaaacttgtatgtatggtggtgtaactgagcataatggaaaccaattagataaatatagaagtattactgttcgggtatttgaagatggtaaaaatttattatcttttgacgtacaaactaataagaaaaaggtgactgctcaagaattagattacctaactcgtcactatttggtgaaaaataaaaaactctatgaatttaacaactcgccttatgaaacgggatatattaaatttatagaaaatgagaatagcttttggtatgacatgatgcctgcaccaggagataaatttgaccaatctaaatatttaatgatgtacaatgacaataaaatggttgattctaaagatgtgaagattgaagtttatcttacgacaaagaaaaag

SEQ ID NO: 9 - protein, 236 aa, Artificial Sequence
  Mutant SEB
ESQPDPKPDELHKSSKFTGLMKVLYDDNHVSAINVKSIDQPLYFDLIYSIKDTKLGNYDNVRVEFKNKDLADKYKDKYVDVFGANYYYQCYFSKKTNDINSHQTDKRKTCMYGGVTEHNGNQLDKYRSITVRVFEDGKNLLSFDVQTNKKKVTAQELDYLTRHYLVKNKKLYEFNNSPYETGYIKFIENENSFWYDMMPAPGDKFDQSKYLMMYNDNKMVDSKDVKIEVYLTTKKK

SEQ ID NO: 10 - DNA, 708 bp, Artificial Sequence
  Mutant SEB
gagagtcaaccagatcctaaaccagatgagttgcacaaatcgagtaaattcactggtttgatgaaagttttgtatgatgataatcatgtatcagcaataaacgttaaatctatagatcaaccgctatactttgacttaatatattctattaaggacactaagttagggaattatgataatgttcgagtcgaatttaaaaacaaagatttagctgataaatacaaagataaatacgtagatgtgtttggagctaattattattatcaatgttatttttctaaaaaaacgaatgatattaattcgcatcaaactgacaaacgaaaaacttgtatgtatggtggtgtaactgagcataatggaaaccaattagataaatatagaagtattactgttcgggtatttgaagatggtaaaaatttattatcttttgacgtacaaactaataagaaaaaggtgactgctcaagaattagattacctaactcgtcactatttggtgaaaaataaaaaactctatgaatttaacaactcgccttatgaaacgggatatattaaatttatagaaaatgagaatagcttttggtatgacatgatgcctgcaccaggagataaatttgaccaatctaaatatttaatgatgtacaatgacaataaaatggttgattctaaagatgtgaagattgaagtttatcttacgacaaagaaaaag

SEQ ID NO: 11 - protein, 236 aa, Artificial Sequence
  Mutant SEB
ESQPDPKPDELHKSSKFTGLMKVLYDDNHVSAINVKSIDQSLYFDLIYSIKDTKLGNYDNVRVEFKNKDLADKYKDKYVDVFGANYYYQCYFSKKTNDINSHQTDKRKTCMYGGVTEHNGNQLDKYRSITVRVFEDGKNLLSFDVQTNKKKVTAQELDYLTRHYLVKNKKLYEFNNSPYETGYIKFIENENSFWYDMMPAPGDKFDQSKYLMMYNDNKMVDSKDVKIEVYLTTKKK

SEQ ID NO: 12 - DNA, 708 bp, Artificial Sequence
  Mutant SEB
gagagtcaaccagatcctaaaccagatgagttgcacaaatcgagtaaattcactggtttgatgaaagttttgtatgatgataatcatgtatcagcaataaacgttaaatctatagatcaaagcctatactttgacttaatatattctattaaggacactaagttagggaattatgataatgttcgagtcgaatttaaaaacaaagatttagctgataaatacaaagataaatacgtagatgtgtttggagctaattattattatcaatgttatttttctaaaaaaacgaatgatattaattcgcatcaaactgacaaacgaaaaacttgtatgtatggtggtgtaactgagcataatggaaaccaattagataaatatagaagtattactgttcgggtatttgaagatggtaaaaatttattatcttttgacgtacaaactaataagaaaaaggtgactgctcaagaattagattacctaactcgtcactatttggtgaaaaataaaaaactctatgaatttaacaactcgccttatgaaacgggatatattaaatttatagaaaatgagaatagcttttggtatgacatgatgcctgcaccaggagataaatttgaccaatctaaatatttaatgatgtacaatgacaataaaatggttgattctaaagatgtgaagattgaagtttatcttacgacaaagaaaaag

SEQ ID NO: 13 - protein, 474 aa, Artificial Sequence
  Mutant SEB
ESQPDPKPDELHKSSKFTGLMKVLYDDNHVSAINVKSIDQFRYFDLIYSIKDTKLGNYDNVRVEFKNKDLADKYKDKYVDVFGANYYYQCYFSKKTNDINSHQTDKRKTCMYGGVTEHNGNQLDKYRSITVRVFEDGKNLLSFDVQTNKKKVTAQELDYLTRHYLVKNKKLYEFNNSPYETGYIKFIENENSFWYDMMPAPGDKFDQSKYLMMYNDNKMVDSKDVKIEVYLTTKKKKLESQPDPKPDELHKSSKFTGLMKVLYDDNHVSAINVKSIDQFRYFDLIYSIKDTKLGNYDNVRVEFKNKDLADKYKDKYVDVFGANYYYQCYFSKKTNDINSHQTDKRKTCMYGGVTEHNGNQLDKYRSITVRVFEDGKNLLSFDVQTNKKKVTAQELDYLTRHYLVKNKKLYEFNNSPYETGYIKFIENENSFWYDMMPAPGDKFDQSKYLMMYNDNKMVDSKDVKIEVYLTTKKK

SEQ ID NO: 14 - DNA, 1422 bp, Artificial Sequence
  Mutant SEB
gagagtcaaccagatcctaaaccagatgagttgcacaaatcgagtaaattcactggtttgatgaaagttttgtatgatgataatcatgtatcagcaataaacgttaaatctatagatcaatttagatactttgacttaatatattctattaaggacactaagttagggaattatgataatgttcgagtcgaatttaaaaacaaagatttagctgataaatacaaagataaatacgtagatgtgtttggagctaattattattatcaatgttatttttctaaaaaaacgaatgatattaattcgcatcaaactgacaaacgaaaaacttgtatgtatggtggtgtaactgagcataatggaaaccaattagataaatatagaagtattactgttcgggtatttgaagatggtaaaaatttattatcttttgacgtacaaactaataagaaaaaggtgactgctcaagaattagattacctaactcgtcactatttggtgaaaaataaaaaactctatgaatttaacaactcgccttatgaaacgggatatattaaatttatagaaaatgagaatagcttttggtatgacatgatgcctgcaccaggagataaatttgaccaatctaaatatttaatgatgtacaatgacaataaaatggttgattctaaagatgtgaagattgaagtttatcttacgacaaagaaaaagaagcttgagagtcaaccagatcctaaaccagatgagttgcacaaatcgagtaaattcactggtttgatgaaagttttgtatgatgataatcatgtatcagcaataaacgttaaatctatagatcaatttagatactttgacttaatatattctattaaggacactaagttagggaattatgataatgttcgagtcgaatttaaaaacaaagatttagctgataaatacaaagataaatacgtagatgtgtttggagctaattattattatcaatgttatttttctaaaaaaacgaatgatattaattcgcatcaaactgacaaacgaaaaacttgtatgtatggtggtgtaactgagcataatggaaaccaattagataaatatagaagtattactgttcgggtatttgaagatggtaaaaatttattatcttttgacgtacaaactaataagaaaaaggtgactgctcaagaattagattacctaactcgtcactatttggtgaaaaataaaaaactctatgaatttaacaactcgccttatgaaacgggatatattaaatttatagaaaatgagaatagcttttggtatgacatgatgcctgcaccaggagataaatttgaccaatctaaatatttaatgatgtacaatgacaataaaatggttgattctaaagatgtgaagattgaagtttatcttacgacaaagaaaaag

SEQ ID NO: 15 - protein, 239 aa, Artificial Sequence
  Mutant SEB
ESQPDPKPDELHKSSKFTGLMENMKVLYDDNHVSAINVKSIDQFRYFDLIYSIKDTKLGNYDNVRVEFKNKDLADKYKDKYVDVFGANYYYQCYFSKKTNDINSHQTDKRKTCMYGGVTEHNGNQLDKYRSITVRVFEDGKNLLSFDVQTNKKKVTAQELDYLTRHYLVKNKKLYEFNNSPYETGYIKFIENENSFWYDMMPAPGDKFDQSKYLMMYNDNKMVDSKDVKIEVYLTTKKK

SEQ ID NO: 16 - DNA, 717 bp, Artificial Sequence
  Mutant SEB
gagagtcaaccagatcctaaaccagatgagttgcacaaatcgagtaaattcactggtttgatggaaaatatgaaagttttgtatgatgataatcatgtatcagcaataaacgttaaatctatagatcaatttagatactttgacttaatatattctattaaggacactaagttagggaattatgataatgttcgagtcgaatttaaaaacaaagatttagctgataaatacaaagataaatacgtagatgtgtttggagctaattattattatcaatgttatttttctaaaaaaacgaatgatattaattcgcatcaaactgacaaacgaaaaacttgtatgtatggtggtgtaactgagcataatggaaaccaattagataaatatagaagtattactgttcgggtatttgaagatggtaaaaatttattatcttttgacgtacaaactaataagaaaaaggtgactgctcaagaattagattacctaactcgtcactatttggtgaaaaataaaaaactctatgaatttaacaactcgccttatgaaacgggatatattaaatttatagaaaatgagaatagcttttggtatgacatgatgcctgcaccaggagataaatttgaccaatctaaatatttaatgatgtacaatgacaataaaatggttgattctaaagatgtgaagattgaagtttatcttacgacaaagaaaaag

SEQ ID NO: 17 - protein, 239 aa, Staphylococcus aureus
ESQPDPKPDELHKASKFTGLMENMKVLYDDNHVSAINVKSIDQFLYFDLIYSIKDTKLGNYDNVRVEFKNKDLADKYKDKYVDVFGANYYYQCYFSKKTNDINSHQTDKRKTCMYGGVTEHNGNQLDKYRSITVRVFEDGKNLLSFDVQTNKKKVTAQELDYLTRHYLVKNKKLYEFNNSPYETGYIKFIENENSFWYDMMPAPGDKFDQSKYLMMYNDNKMVDSKDVKIEVYLTTKKK

SEQ ID NO: 18 - DNA, 717 bp, Staphylococcus aureus
gagagtcaaccagatcctaaaccagatgagttgcacaaagcgagtaaattcactggtttgatggaaaatatgaaagttttgtatgatgataatcatgtatcagcaataaacgttaaatctatagatcaatttctatactttgacttaatatattctattaaggacactaagttagggaattatgataatgttcgagtcgaatttaaaaacaaagatttagctgataaatacaaagataaatacgtagatgtgtttggagctaattattactatcaatgttatttttctaaaaaaacgaatgatattaattcacatcaaactgacaaacgaaaaacttgtatgtatggtggtgtaactgagcataatggaaaccaattagataaatatagaagtattactgttcgggtatttgaagatggtaaaaatttattatcttttgacgtacaaactaataagaaaaaagtgactgctcaagaattagattacctaactcgtcactatttggtgaaaaataaaaaactctatgaatttaacaactcgccttatgaaacgggatatattaaatttatagaaaatgagaatagcttttggtatgacatgatgcctgcaccaggagataaatttgaccaatctaaatatttaatgatgtacaatgacaataaaatggttgattctaaagatgtgaagattgaagtttatcttacgacaaagaaaaag

SEQ ID NO: 19 - protein, 239 aa, Staphylococcus aureus
ESQPDPKPDELHKSSKFTGLMENMKVLYDDNHVSAINVKSIDQFLYFDLIYSIKDTKLGNYDNVRVEFKNKDLADKYKDKYVDVFGANYYYQCYFSKKTNDINSHQTDKRKTCMYGGVTEHNGNQLDKYRSISVRVFEDGKNLLSFDVQTNKKKVTAQELDYLTRHYLVKNKKLYEFNNSPYETGYIKFIENENSFWYDMMPAPGDKFDQSKYLMMYNDNKMVDSKDVKIEVYLTTKKK

SEQ ID NO: 20 - DNA, 717 bp, Staphylococcus aureus
gagagtcaaccagatcctaaaccagatgagttgcacaaatcgagtaaattcactggtttgatggaaaatatgaaagttttgtatgatgataatcatgtatcagcaataaacgttaaatctatagatcaatttctatactttgacttaatatattctattaaggacactaagttagggaattatgataatgttcgagtcgaatttaaaaacaaagatttagctgataaatacaaagataaatacgtagatgtgtttggagctaattattattatcaatgttatttttctaaaaaaacgaatgatattaattcgcatcaaactgacaaacgaaaaacttgtatgtatggtggtgtaactgagcataatggaaaccaattagataaatatagaagtatttctgttcgggtatttgaagatggtaaaaatttattatcttttgacgtacaaactaataagaaaaaggtgactgctcaagaattagattacctaactcgtcactatttggtgaaaaataaaaaactctatgaatttaacaactcgccttatgaaacgggatatattaaatttatagaaaatgagaatagcttttggtatgacatgatgcctgcaccaggagataaatttgaccaatctaaatatttaatgatgtacaatgacaataaaatggttgattctaaagatgtgaagattgaagtttatcttacgacaaagaaaaag

SEQ ID NO: 21 - protein, 239 aa, Staphylococcus aureus
ESQPDPKPDELHKSSKFTGLMENMKVLYDDNHVSAINVKSIDQFLYFDLIYSIKDTKLGNYDNVRVEFKNKDLADKYKDKYLDVFGANYYYQCYFSKKTNDINSHQTDKRKTCMYGGVTEHNGNQLDKYRSITVRVFEDGKNLLSFDVQTNKKKVTAQELDYLTRHYLVKNKKLYEFNNSPYETGYIKFIENENSFWYDMMPAPGDKFDQSKYLMMYNDNKMVDSKDVKIEVYLTTKKK

SEQ ID NO: 22 - DNA, 717 bp, Staphylococcus aureus
gagagtcaaccagatcctaaaccagatgagttgcacaaatcgagtaaattcactggtttgatggaaaatatgaaagttttgtatgatgataatcatgtatcagcaataaacgttaaatctatagatcaatttctatactttgacttaatatattctattaaggacactaagttagggaattatgataatgttcgagtcgaatttaaaaacaaagatttagctgataaatacaaagataaatacttagatgtgtttggagctaattattattatcaatgttatttttctaaaaaaacgaatgatattaattcgcatcaaactgacaaacgaaaaacttgtatgtatggtggtgtaactgagcataatggaaaccaattagataaatatagaagtattactgttcgggtatttgaagatggtaaaaatttattatcttttgacgtacaaactaataagaaaaaggtgactgctcaagaattagattacctaactcgtcactatttggtgaaaaataaaaaactctatgaatttaacaactcgccttatgaaacgggatatattaaatttatagaaaatgagaatagcttttggtatgacatgatgcctgcaccaggagataaatttgaccaatctaaatatttaatgatgtacaatgacaataaaatggttgattctaaagatgtgaagattgaagtttatcttacgacaaagaaaaag

SEQ ID NO: 23 - protein, 239 aa, Staphylococcus aureus
ESQPDPKPDELHKSSKFTGLMENMKVLYDDNHVSAINVKSIDQFLYFDLIYSIKDTKLGNYDNVRVEFKNKDLADKYKDKYVDVFGANYYYQCYFSKKTNDINSHQTDKRKTCMYGGVTEHNGNQLDKYRSITVRVFEDGENLLSFDVQTNKKKVTAQELDYLTRHYLVKNKKLYEFNNSPYETGYIKFIENENSFWYDMMPAPGDKFDQSKYLMMYNDNKMVDSKDVKIEVYLTTKKK

SEQ ID NO: 24 - DNA, 717 bp, Staphylococcus aureus
gagagtcaaccagatcctaaaccagatgagttgcacaaatcgagtaaattcactggtttgatggaaaatatgaaagttttgtatgatgataatcatgtatcagcaataaacgttaaatctatagatcaatttctatactttgacttaatatattctattaaggacactaagttagggaattatgataatgttcgagtcgaatttaaaaacaaagatttagctgataaatacaaagataaatacgtagatgtgtttggagctaattattattatcaatgttatttttctaaaaaaacgaatgatattaattcgcatcaaactgacaaacgaaaaacttgtatgtatggtggtgtaactgagcataatggaaaccaattagataaatatagaagtattactgttcgggtatttgaagatggtgaaaatttattatcttttgacgtacaaactaataagaaaaaggtgactgctcaagaattagattacctaactcgtcactatttggtgaaaaataaaaaactctatgaatttaacaactcgccttatgaaacgggatatattaaatttatagaaaatgagaatagcttttggtatgacatgatgcctgcaccaggagataaatttgaccaatctaaatatttaatgatgtacaatgacaataaaatggttgattctaaagatgtgaagattgaagtttatcttacgacaaagaaaaag

SEQ ID NO: 25 - protein, 239 aa, Staphylococcus aureus
ESQPDPKPDELHKSSKFTGLMENMKVLYDDNHVSAINVKSIDQFLYFDLIYSIKDTKLGNYDNVRVEFKNKDLADKYKDKYVDVFGANYYYQCYFSKKTNDINSHQTDKRKTCMYGGVTEHNGNQLDKYRSITVRVFEDGKNLLSFDVQINKKKVTAQELDYLTRHYLVKNKKLYEFNNSPYETGYIKFIENENSFWYDMMPAPGDKFDQSKYLMMYNDNKMVDSKDVKIEVYLTTKKK

SEQ ID NO: 26 - DNA, 717 bp, Staphylococcus aureus
gagagtcaaccagatcctaaaccagatgagttgcacaaatcgagtaaattcactggtttgatggaaaatatgaaagttttgtatgatgataatcatgtatcagcaataaacgttaaatctatagatcaatttctatactttgacttaatatattctattaaggacactaagttagggaattatgataatgttcgagtcgaatttaaaaacaaagatttagctgataaatacaaagataaatacgtagatgtgtttggagctaattattattatcaatgttatttttctaaaaaaacgaatgatattaattcgcatcaaactgacaaacgaaaaacttgtatgtatggtggtgtaactgagcataatggaaaccaattagataaatatagaagtattactgttcgggtatttgaagatggtaaaaatttattatcttttgacgtacaaattaataagaaaaaggtgactgctcaagaattagattacctaactcgtcactatttggtgaaaaataaaaaactctatgaatttaacaactcgccttatgaaacgggatatattaaatttatagaaaatgagaatagcttttggtatgacatgatgcctgcaccaggagataaatttgaccaatctaaatatttaatgatgtacaatgacaataaaatggttgattctaaagatgtgaagattgaagtttatcttacgacaaagaaaaag

SEQ ID NO: 27 - protein, 239 aa, Staphylococcus aureus
ESQPDPNPDELHKSSKFTGLMENMKVLYDDNHVSAINVKSIDQFLYFDLIYSIKDTKLGNYDNVRVEFKNKDLADKYKDKYVDVFGANYYYQCYFSKKTNDINSHQTDKRKTCMYGGVTEHNGNQLDKYRSITVRVFEDGKNLLSFDVQTNKKKVTAQELDYLTRHYLVKNKKLYEFNNSPYETGYIKFIENENSFWYDMMPAPGDKFDQSKYLMMYNDNKMVDSKDVKIEVYLTTKKK

SEQ ID NO: 28 - DNA, 717 bp, Staphylococcus aureus
gagagtcaaccagatcctaatccagatgagttgcacaaatcgagtaaattcactggtttgatggaaaatatgaaagttttgtatgatgataatcatgtatcagcaataaacgttaaatctatagatcaatttctatactttgacttaatatattctattaaggacactaagttagggaattatgataatgttcgagtcgaatttaaaaacaaagatttagctgataaatacaaagataaatacgtagatgtgtttggagctaattattattatcaatgttatttttctaaaaaaacgaatgatattaattcgcatcaaactgacaaacgaaaaacttgtatgtatggtggtgtaactgagcataatggaaaccaattagataaatatagaagtattactgttcgggtatttgaagatggtaaaaatttattatcttttgatgtacaaactaataagaaaaaggtgactgctcaagaattagattacctaactcgtcactatttggtgaaaaataaaaaactctatgaatttaacaactcgccttatgaaacgggatatattaaatttatagaaaatgagaatagcttttggtatgacatgatgcctgcaccaggagataaatttgaccaatctaaatatttaatgatgtacaatgacaataaaatggttgattctaaagatgtgaagattgaagtttatcttacgacaaagaaaaag

SEQ ID NO: 29 - protein, 239 aa, Staphylococcus aureus
ESQPDPKPDELHKSSKFTGLMENMKVLYDDNHVSAINVKSIDQFLYFDLIYSIKDTKLGNYDNVRVEFKNKDLADKYKDKYVDVFGANYYYQCYFSKKTNDINSHQTDKRKTCMYGGVTEHNGNQLDKYRSITVRVFEDGKNLLSFDVQTNKKKVTAQELDYLTRHYLVKNKKLYEFNNSPYETGYIKFIENENSFWYDMMPAPGDKFDQSKYLMMYNDNKMVDFKDVKIEVYLTTKKK

SEQ ID NO: 30 - DNA, 717 bp, Staphylococcus aureus
gagagtcaaccagatcctaaaccagatgagttgcacaaatcgagtaaattcactggtttgatggaaaatatgaaagttttgtatgatgataatcatgtatcagcaataaacgttaaatctatagatcaatttctatactttgacttaatatattctattaaggacactaagttagggaattatgataatgttcgagtcgaatttaaaaacaaagatttagctgataaatacaaagataaatacgtagatgtgtttggagctaattattattatcaatgttatttttctaaaaaaacgaatgatattaattcgcatcaaactgacaaacgaaaaacttgtatgtatggtggtgtaactgagcataatggaaaccaattagataaatatagaagtattactgttcgggtatttgaagatggtaaaaatttattatcttttgacgtacaaactaataagaaaaaggtgactgctcaagaattagattacctaactcgtcactatttggtgaaaaataaaaaactctatgaatttaacaactcgccttatgaaacgggatatattaaatttatagaaaatgagaatagcttttggtatgacatgatgcctgcaccaggagataaatttgaccaatctaaatatttaatgatgtacaatgacaataaaatggttgattttaaagatgtgaagattgaagtttatcttacgacaaagaaaaag

SEQ ID NO: 31 - protein, 474 aa, Artificial Sequence
  Mutant SEB
ESQPDPKPDELHKSSKFTGLMKVLYDDNHVSAINVKSIDQFRYFDLIYSIKDTKLGNYDNVRVEFKNKDLADKYKDKYVDVFGANYYYQCYFSKKTNDINSHQTDKRKTCMYGGVTEHNGNQLDKYRSITVRVFEDGKNLLSFDVQTNKKKVTAQELDYLTRHYLVKNKKLYEFNNSPYETGYIKFIENENSFWYDMMPAPGDKFDQSKYLMMYNDNKMVDSKDVKIEVYLTTKKKHMESQPDPKPDELHKSSKFTGLMKVLYDDNHVSAINVKSIDQFRYFDLIYSIKDTKLGNYDNVRVEFKNKDLADKYKDKYVDVFGANYYYQCYFSKKTNDINSHQTDKRKTCMYGGVTEHNGNQLDKYRSITVRVFEDGKNLLSFDVQTNKKKVTAQELDYLTRHYLVKNKKLYEFNNSPYETGYIKFIENENSFWYDMMPAPGDKFDQSKYLMMYNDNKMVDSKDVKIEVYLTTKKK

SEQ ID NO: 32 - DNA, 1422 bp, Artificial Sequence
  Mutant SEB
atgatgataatcatgtatcagcaataaacgttaaatctatagatcaatttagatactttgacttaatatattctagagagtcaaccagatcctaaaccagatgagttgcacaaatcgagtaaattcactggtttgatgaaagttttgtttaaggacactaagttagggaattatgataatgttcgagtcgaatttaaaaacaaagatttagctgataaatacaaagataaatacgtagatgtgtttggagctaattattattatcaatgttatttttctaaaaaaacgaatgatattaattcgcatcaaactgacaaacgaaaaacttgtatgtatggtggtgtaactgagcataatggaaaccaattagataaatatagaagtattactgttcgggtatttgaagatggtaaaaatttattatcttttgacgtacaaactaataagaaaaaggtgactgctcaagaattagattacctaactcgtcactatttggtgaaaaataaaaaactctatgaatttaacaactcgccttatgaaacgggatatattaaatttatagaaaatgagaatagcttttggtatgacatgatgcctgcaccaggagataaatttgaccaatctaaatatttaatgatgtacaatgacaataaaatggttgattctaaagatgtgaagattgaagtttatcttacgacaaagaaaaagcatatggagagtcaaccagatcctaaaccagatgagttgcacaaatcgagtaaattcactggtttgatgaaagttttgtatgatgataatcatgtatcagcaataaacgttaaatctatagatcaatttagatactttgacttaatatattctattaaggacactaagttagggaattatgataatgttcgagtcgaatttaaaaacaaagatttagctgataaatacaaagataaatacgtagatgtgtttggagctaattattattatcaatgttatttttctaaaaaaacgaatgatattaattcgcatcaaactgacaaacgaaaaacttgtatgtatggtggtgtaactgagcataatggaaaccaattagataaatatagaagtattactgttcgggtatttgaagatggtaaaaatttattatcttttgacgtacaaactaataagaaaaaggtgactgctcaagaattagattacctaactcgtcactatttggtgaaaaataaaaaactctatgaatttaacaactcgccttatgaaacgggatatattaaatttatagaaaatgagaatagcttttggtatgacatgatgcctgcaccaggagataaatttgaccaatctaaatatttaatgatgtacaatgacaataaaatggttgattctaaagatgtgaagattgaagtttatcttacgacaaagaaaaag

SEQ ID NO: 33 - protein, 474 aa, Artificial Sequence
  Mutant SEB
ESQPDPKPDELHKSSKFTGLMKVLYDDNHVSAINVKSIDQFRYFDLIYSIKDTKLGNYDNVRVEFKNKDLADKYKDKYVDVFGANYYYQCYFSKKTNDINSHQTDKRKTCMYGGVTEHNGNQLDKYRSITVRVFEDGKNLLSFDVQTNKKKVTAQELDYLTRHYLVKNKKLYEFNNSPYETGYIKFIENENSFWYDMMPAPGDKFDQSKYLMMYNDNKMVDSKDVKIEVYLTTKKKGTESQPDPKPDELHKSSKFTGLMKVLYDDNHVSAINVKSIDQFRYFDLIYSIKDTKLGNYDNVRVEFKNKDLADKYKDKYVDVFGANYYYQCYFSKKTNDINSHQTDKRKTCMYGGVTEHNGNQLDKYRSITVRVFEDGKNLLSFDVQTNKKKVTAQELDYLTRHYLVKNKKLYEFNNSPYETGYIKFIENENSFWYDMMPAPGDKFDQSKYLMMYNDNKMVDSKDVKIEVYLTTKKK

SEQ ID NO: 34 - DNA, 1422 bp, Artificial Sequence
  Mutant SEB
gagagtcaaccagatcctaaaccagatgagttgcacaaatcgagtaaattcactggtttgatgaaagttttgtatgatgataatcatgtatcagcaataaacgttaaatctatagatcaatttagatactttgacttaatatattctattaaggacactaagttagggaattatgataatgttcgagtcgaatttaaaaacaaagatttagctgataaatacaaagataaatacgtagatgtgtttggagctaattattattatcaatgttatttttctaaaaaaacgaatgatattaattcgcatcaaactgacaaacgaaaaacttgtatgtatggtggtgtaactgagcataatggaaaccaattagataaatatagaagtattactgttcgggtatttgaagatggtaaaaatttattatcttttgacgtacaaactaataagaaaaaggtgactgctcaagaattagattacctaactcgtcactatttggtgaaaaataaaaaactctatgaatttaacaactcgccttatgaaacgggatatattaaatttatagaaaatgagaatagcttttggtatgacatgatgcctgcaccaggagataaatttgaccaatctaaatatttaatgatgtacaatgacaataaaatggttgattctaaagatgtgaagattgaagtttatcttacgacaaagaaaaagggtaccgagagtcaaccagatcctaaaccagatgagttgcacaaatcgagtaaattcactggtttgatgaaagttttgtatgatgataatcatgtatcagcaataaacgttaaatctatagatcaatttagatactttgacttaatatattctattaaggacactaagttagggaattatgataatgttcgagtcgaatttaaaaacaaagatttagctgataaatacaaagataaatacgtagatgtgtttggagctaattattattatcaatgttatttttctaaaaaaacgaatgatattaattcgcatcaaactgacaaacgaaaaacttgtatgtatggtggtgtaactgagcataatggaaaccaattagataaatatagaagtattactgttcgggtatttgaagatggtaaaaatttattatcttttgacgtacaaactaataagaaaaaggtgactgctcaagaattagattacctaactcgtcactatttggtgaaaaataaaaaactctatgaatttaacaactcgccttatgaaacgggatatattaaatttatagaaaatgagaatagcttttggtatgacatgatgcctgcaccaggagataaatttgaccaatctaaatatttaatgatgtacaatgacaataaaatggttgattctaaagatgtgaagattgaagtttatcttacgacaaagaaaaag

SEQ ID NO: 35 - protein, 476 aa, Artificial Sequence
  Mutant SEB
ESQPDPKPDELHKSSKFTGLMKVLYDDNHVSAINVKSIDQFRYFDLIYSIKDTKLGNYDNVRVEFKNKDLADKYKDKYVDVFGANYYYQCYFSKKTNDINSHQTDKRKTCMYGGVTEHNGNQLDKYRSITVRVFEDGKNLLSFDVQTNKKKVTAQELDYLTRHYLVKNKKLYEFNNSPYETGYIKFIENENSFWYDMMPAPGDKFDQSKYLMMYNDNKMVDSKDVKIEVYLTTKKKGGGSESQPDPKPDELHKSSKFTGLMKVLYDDNHVSAINVKSIDQFRYFDLIYSIKDTKLGNYDNVRVEFKNKDLADKYKDKYVDVFGANYYYQCYFSKKTNDINSHQTDKRKTCMYGGVTEHNGNQLDKYRSITVRVFEDGKNLLSFDVQTNKKKVTAQELDYLTRHYLVKNKKLYEFNNSPYETGYIKFIENENSFWYDMMPAPGDKFDQSKYLMMYNDNKMVDSKDVKIEVYLTTKKK

SEQ ID NO: 36 - DNA, 1428 bp, Artificial Sequence
  Mutant SEB
gagagtcaaccagatcctaaaccagatgagttgcacaaatcgagtaaattcaccggtttgatgaaagttttgtatgatgataatcatgtatcagcaataaacgttaaatctatagatcaatttagatactttgacttaatatattctattaaggacactaagttagggaattatgataatgttcgagtcgaatttaaaaacaaagatttagctgataaatacaaagataaatacgtagatgtgtttggagctaattattattatcaatgttatttttctaaaaaaacgaatgatattaattcgcatcaaactgacaaacgaaaaacttgtatgtatggtggtgtaactgagcataatggaaaccaattagataaatatagaagtattactgttcgggtatttgaagatggtaaaaatttattatcttttgacgtacaaactaataagaaaaaggtgactgctcaagaattagattacctaactcgtcactatttggtgaaaaataaaaaactctatgaatttaacaactcgccttatgaaacgggatatattaaatttatagaaaatgagaatagcttttggtatgacatgatgcctgcaccaggagataaatttgaccaatctaaatatttaatgatgtacaatgacaataaaatggttgattctaaagatgtgaagattgaagtttatcttacgacaaagaaaaagggcggtggatccgagagtcaaccagatcctaaaccagatgagttgcacaaatcgagtaaattcactggtttgatgaaagttttgtatgatgataatcatgtatcagcaataaacgttaaatctatagatcaatttagatactttgacttaatatattctattaaggacactaagttagggaattatgataatgttcgagtcgaatttaaaaacaaagatttagctgataaatacaaagataaatacgtagatgtgtttggagctaattattattatcaatgttatttttctaaaaaaacgaatgatattaattcgcatcaaactgacaaacgaaaaacttgtatgtatggtggtgtaactgagcataatggaaaccaattagataaatatagaagtattactgttcgggtatttgaagatggtaaaaatttattatcttttgacgtacaaactaataagaaaaaggtgactgctcaagaattagattacctaactcgtcactatttggtgaaaaataaaaaactctatgaatttaacaactcgccttatgaaacgggatatattaaatttatagaaaatgagaatagcttttggtatgacatgatgcctgcaccaggagataaatttgaccaatctaaatatttaatgatgtacaatgacaataaaatggttgattctaaagatgtgaagattgaagtttatcttacgacaaagaaaaag

SEQ ID NO: 37 - protein, 5 aa, Binding region
MENMK

SEQ ID NO: 38 - protein, 6 aa, Artificial Sequence
  binding region
DQFLYF